European Patent Specification EP 3 768 726 B1, published October 30, 2024. Title: DUAL SPECIFICITY ANTIBODIES TO PD-L1 AND PD-L2 AND METHODS OF USE THEREFOR. Applicant: Board of Regents, The University of Texas System et al. Application Not yet assigned. The sequence listing filed with the application follows.

SEQUENCE LISTING (42 sequences)

SEQ ID NO: 1 - protein, 290 aa, Homo sapiens
MRIFAVFIFMTYWHLLNAFTVTVPKDLYVVEYGSNMTIECKFPVEKQLDLAALIVYWEMEDKNIIQFVHGEEDLKVQHSSYRQRARLLKDQLSLGNAALQITDVKLQDAGVYRCMISYGGADYKRITVKVNAPYNKINQRILVVDPVTSEHELTCQAEGYPKAEVIWTSSDHQVLSGKTTTTNSKREEKLFNVTSTLRINTTTNEIFYCTFRRLDPEENHTAELVIPELPLAHPPNERTHLVILGAILLCLGVALTFIFRLRKGRMMDVKKCGIQDTNSKKQSDTHLEET

SEQ ID NO: 2 - protein, 273 aa, Homo sapiens
MIFLLLMLSLELQLHQIAALFTVTVPKELYIIEHGSNVTLECNFDTGSHVNLGAITASLQKVENDTSPHRERATLLEEQLPLGKASFHIPQVQVRDEGQYQCIIIYGVAWDYKYLTLKVKASYRKINTHILKVPETDEVELTCQATGYPLAEVSWPNVSVPANTSHSRTPEGLYQVTSVLRLKPPPGRNFSCVFWNTHVRELTLASIDLQSQMEPRTHPTWLLHIFIPFCIIAFIFIATVIALRKQLCQKLYSSKDTTKRPVTTTKREVNSAI

SEQ ID NO: 3 - DNA, 354 bp, Homo sapiens
caggtgcagctggtgcagtctggggctgaggtgaagaagcctggggcctcagtgaaggtctcctgcaaggcttctggaggcaccttccgtagctatgctatccagtgggtgcgacaggcccctggacaagggcttgagtggatgggatggatcatccctggttttggtacagcaaactacgcacagaagttccagggcagagtcacgattaccgcggacgaatccacgagcacagcctacatggagctgagcagcctgagatctgaggacacggcggtgtactactgcgccagagagttgtcccacggtggtctcagttactggggacagggtacattggtcaccgtctcctca

SEQ ID NO: 4 - DNA, 321 bp, Homo sapiens
gacatccagatgacccagtctccatcttccgtgtctgcatctgtaggagacagagtcaccatcacttgtcgggcgagtcagggtattagcagctggttagcctggtatcagcagaaaccagggaaagcccctaagctcctgatctatgctgcatccagtttgcaaagtggggtcccatcaaggttcagcggcagtggatctgggacagatttcactctcaccatcagcagcctgcagcctgaagattttgcaacttactattgtcaacaggctaacagtttccctatcacctttggcggagggaccaaggttgagatcaaa

SEQ ID NO: 5 - DNA, 354 bp, Homo sapiens
caggtgcagctggtgcagtctggggctgaggtgaagaagcctgggtcctcggtgaaggtctcctgcaaggcttctggaggcaccttcagcagctattttatctcgtgggtgcgacaggcccctggacaagggcttgagtggatgggacagatcatccctaatgtgggtacagcaaactacgcacagaagttccagggcagagtcacgattaccgcggacgaatccacgagcacagcctacatggagctgagcagcctgagatctgaggacacggcggtgtactactgcgccagggaccagaccgctaaggcacacctggtctggggacagggtacattggtcaccgtctcctca

SEQ ID NO: 6 - DNA, 321 bp, Homo sapiens
gacatccagatgacccagtctccttccaccctgtctgcatctgtaggagacagagtcaccatcacttgccgggccagtcagagtattagtagctggttggcctggtatcagcagaaaccagggaaagcccctaagctcctgatctataaagcctccagtttggaaagtggggtcccatcaaggttcagcggcagtggatctgggacagaattcactctcaccatcagcagcctgcagcctgatgattttgcaacttattactgccaacagtataatagttatcctatcacctttggcggagggaccaaggttgagatcaaa

SEQ ID NO: 7 - DNA, 360 bp, Homo sapiens
caggtgcagctggtgcagtctggggctgaggtgaagaagcctgggtcctcggtgaaggtctcctgcaaggcttctggaggcaccttctcgagccatgctatcagctgggtgcgacaggcccctggacaagggcttgagtggatgggagggatcatccctatctttggttgggcattgtacgcacagaagttccagggcagagtcacgattaccgcggacgaatccacgagcacagcctacatggagctgagcagcctgagatctgaggacacggcggtgtactactgcgccagaccaggagaccacagagcttcccatttcgattactggggacagggtacattggtcaccgtctcctca

SEQ ID NO: 8 - DNA, 321 bp, Homo sapiens; identical to SEQ ID NO: 4

SEQ ID NO: 9 - DNA, 360 bp, Homo sapiens
caggtgcagctggtgcagtctggggctgaggtgaagaagcctgggtcctcggtgaaggtctcctgcaaggcttctggaggcaccttcagcgagtatgctatcgtgtgggtgcgacaggcccctggacaagggcttgagtggatgggagggatcatccctctgtttggtacagcaaactacgcacagaagttccagggcagagtcacgattaccgcggacgaatccacgagcacagcctacatggagctgagcagcctgagatctgaggacacggcggtgtactactgcgccagaccgttggaccgcagaatagtagcattcgacatatggggtcagggtacaatggtcaccgtctcctca

SEQ ID NO: 10 - DNA, 321 bp, Homo sapiens; identical to SEQ ID NO: 6

SEQ ID NO: 11 - protein, 118 aa, Homo sapiens
QVQLVQSGAEVKKPGASVKVSCKASGGTFRSYAIQWVRQAPGQGLEWMGWIIPGFGTANYAQKFQGRVTITADESTSTAYMELSSLRSEDTAVYYCARELSHGGLSYWGQGTLVTVSS

SEQ ID NO: 12 - protein, 107 aa, Homo sapiens
DIQMTQSPSSVSASVGDRVTITCRASQGISSWLAWYQQKPGKAPKLLIYAASSLQSGVPSRFSGSGSGTDFTLTISSLQPEDFATYYCQQANSFPITFGGGTKVEIK

SEQ ID NO: 13 - protein, 118 aa, Homo sapiens
QVQLVQSGAEVKKPGSSVKVSCKASGGTFSSYFISWVRQAPGQGLEWMGQIIPNVGTANYAQKFQGRVTITADESTSTAYMELSSLRSEDTAVYYCARDQTAKAHLVWGQGTLVTVSS

SEQ ID NO: 14 - protein, 107 aa, Homo sapiens
DIQMTQSPSTLSASVGDRVTITCRASQSISSWLAWYQQKPGKAPKLLIYKASSLESGVPSRFSGSGSGTEFTLTISSLQPDDFATYYCQQYNSYPITFGGGTKVEIK

SEQ ID NO: 15 - protein, 120 aa, Homo sapiens
QVQLVQSGAEVKKPGSSVKVSCKASGGTFSSHAISWVRQAPGQGLEWMGGIIPIFGWALYAQKFQGRVTITADESTSTAYMELSSLRSEDTAVYYCARPGDHRASHFDYWGQGTLVTVSS

SEQ ID NO: 16 - protein, 107 aa, Homo sapiens; identical to SEQ ID NO: 12

SEQ ID NO: 17 - protein, 120 aa, Homo sapiens
QVQLVQSGAEVKKPGSSVKVSCKASGGTFSEYAIVWVRQAPGQGLEWMGGIIPLFGTANYAQKFQGRVTITADESTSTAYMELSSLRSEDTAVYYCARPLDRRIVAFDIWGQGTMVTVSS

SEQ ID NO: 18 - protein, 107 aa, Homo sapiens; identical to SEQ ID NO: 14

SEQ ID NO: 19 - protein, 9 aa, Homo sapiens
GTFRSYAIQ

SEQ ID NO: 20 - protein, 17 aa, Homo sapiens
WIIPGFGTANYAQKFQG

SEQ ID NO: 21 - protein, 11 aa, Homo sapiens
ARELSHGGLSY

SEQ ID NO: 22 - protein, 11 aa, Homo sapiens
RASQGISSWLA

SEQ ID NO: 23 - protein, 7 aa, Homo sapiens
AASSLQS

SEQ ID NO: 24 - protein, 9 aa, Homo sapiens
QQANSFPIT

SEQ ID NO: 25 - protein, 9 aa, Homo sapiens
GTFSSYFIS

SEQ ID NO: 26 - protein, 17 aa, Homo sapiens
QIIPNVGTANYAQKFQG

SEQ ID NO: 27 - protein, 11 aa, Homo sapiens
ARDQTAKAHLV

SEQ ID NO: 28 - protein, 11 aa, Homo sapiens
RASQSISSWLA

SEQ ID NO: 29 - protein, 7 aa, Homo sapiens
KASSLES

SEQ ID NO: 30 - protein, 9 aa, Homo sapiens
QQYNSYPIT

SEQ ID NO: 31 - protein, 9 aa, Homo sapiens
GTFSSHAIS

SEQ ID NO: 32 - protein, 17 aa, Homo sapiens
GIIPIFGWALYAQKFQG

SEQ ID NO: 33 - protein, 13 aa, Homo sapiens
ARPGDHRASHFDY

SEQ ID NO: 34 - protein, 11 aa, Homo sapiens
RASQGISSWLA

SEQ ID NO: 35 - protein, 7 aa, Homo sapiens
AASSLQS

SEQ ID NO: 36 - protein, 9 aa, Homo sapiens
QQANSFPIT

SEQ ID NO: 37 - protein, 9 aa, Homo sapiens
GTFSEYAIV

SEQ ID NO: 38 - protein, 17 aa, Homo sapiens
GIIPLFGTANYAQKFQG

SEQ ID NO: 39 - protein, 13 aa, Homo sapiens
ARPLDRRIVAFDI

SEQ ID NO: 40 - protein, 11 aa, Homo sapiens
RASQSISSWLA

SEQ ID NO: 41 - protein, 7 aa, Homo sapiens
KASSLES

SEQ ID NO: 42 - protein, 9 aa, Homo sapiens
QQYNSYPIT